European Patent Application EP 4 763 993 A1, published June 24, 2026. Title: ARRAYS AND METHODS FOR SPATIAL EPIGENOMIC PROFILING. Applicant: COMMISSARIAT A L'ENERGIE ATOMIQUE ET AUX ENERGIES ALTERNATIVES. Application EP. The sequence listing filed with the application follows.

SEQUENCE LISTING (6 sequences)

SEQ ID NO: 1 - DNA, 19 bp, synthetic construct
  source 1..19: mol_type = other DNA
ctgtctcttatacacatct

SEQ ID NO: 2 - DNA, 26 bp, synthetic construct
  source 1..26: mol_type = other DNA
gactcgtaatacgactcactataggg

SEQ ID NO: 3 - DNA, 30 bp, synthetic construct
  source 1..30: mol_type = other DNA
acattgaagaacctgtagataactcgctgt

SEQ ID NO: 4 - DNA, 35 bp, synthetic construct
  source 1..35: mol_type = other DNA
gttcagacgtgtgctcttccgatctgggggggggh

SEQ ID NO: 5 - DNA, 25 bp, synthetic construct
  source 1..25: mol_type = other DNA
gttcagacgtgtgctcttccgatct

SEQ ID NO: 6 - DNA, 46 bp, synthetic construct
  source 1..46: mol_type = other DNA
tacactctttccctacacgacgctcttccgatctgactcgtaatac